European Patent Application EP 4 497 834 A1, published January 29, 2025. Title: 核酸増幅方法、核酸増幅システム、ウイルス検出方法、及びウイルス検出システム. Applicant: 京セラ株式会社. Application JP. The sequence listing filed with the application follows.

SEQUENCE LISTING (9 sequences)

SEQ ID NO: 1 - DNA, 281 bp, Coronavirus SARS-CoV-2
  source 1..281: mol_type = genomic DNA
ccaagatggtatttctactacctaggaactgggccagaagctggacttccctatggtgctaacaaagacggcatcatatgggttgcaactgagggagccttgaatacaccaaaagatcacattggcacccgcaatcctgctaacaatgctgcaatcgtgctacaacttcctcaaggaacaacattgccaaaaggcttctacgcagaagggagcagaggcggcagtcaagcctcttctcgttcctcatcacgtagtcgcaacagttcaagaaattcaactcc

SEQ ID NO: 2 - DNA, 20 bp, Enterobacteria phage T7
  source 1..20: mol_type = genomic DNA
taatacgactcactataggg

SEQ ID NO: 3 - DNA, 29 bp, Influenza A virus PR8
  source 1..29: mol_type = genomic DNA
ccmaggtcgaaacgtaygttctctctatc

SEQ ID NO: 4 - DNA, 52 bp, Influenza A virus PR8
  source 1..52: mol_type = genomic DNA
taatacgactcactatagggtgacagratyggtcttgtctttagccaytcca

SEQ ID NO: 5 - DNA, 19 bp, Corona virus SARS-CoV-2
  source 1..19: mol_type = genomic DNA
cacattggcacccgcaatc

SEQ ID NO: 6 - DNA, 40 bp, Corona virus SARS-CoV-2
  source 1..40: mol_type = genomic DNA
taatacgactcactataggggaggaacgagaagaggcttg

SEQ ID NO: 7 - DNA, 27 bp, Influenza A virus PR8
  source 1..27: mol_type = genomic DNA
ccaagcccctcaaagccgagagcttgg

SEQ ID NO: 8 - DNA, 27 bp, Influenza A virus PR8
  source 1..27: mol_type = genomic DNA
ccaagcccctcaaagccgagagcttgg

SEQ ID NO: 9 - DNA, 37 bp, Coronavirus SARS-CoV-2
  source 1..37: mol_type = genomic DNA
ccaagcacttcctcaaggaacaacattgccagcttgg